European Patent Specification EP 3 490 612 B1, published August 21, 2024. Title: METHODS FOR GYNECOLOGIC NEOPLASM DIAGNOSIS. Applicant: Lai Hung-Cheng. The sequence listing filed with the application follows.

SEQUENCE LISTING (13 sequences)

SEQ ID NO: 1 - DNA, 3199 bp, Homo sapiens
cgtctacgtagtatttctgtccccggaagactggatctcagggaattattatggaagatactgctgagcccctttcatcctttccaggtgaaaatacagacatttttgtgtcgccctcacccttcctttatgaaataaggtgcccaactgttctgatattaccattcaaaaacaggttctgtggcgaacctcatttgtgaatctattacagagattaatagattatttctcctttttcaactaattctcagtggggaaatttaaccatatggtaaggagagaattagaatttcatcacattagagcaaaatgtaatgaaaagagtccaacacctggggccaactccgaaagccacaattaaaaggtttttaatgaaaccagagaaaccaaaaattgcatagtcttcagtacttctgccatataagaaagagttattggaaggtgttgggaaatattgtttttacttatgtcataaggatgaaaaccagctgctaaataccatgtgtacccagagaccgaactcaggagtgagatgaccgcgtgtaccagtgcccatccggagaggagcacttgtttttacattctcccttcccgaaccctccaagaacaaccgaggctgatccagatgtccttaaatggcttccgggtaaataaatatgcataaatgcctcacttcgtgtgggagcggatttgactcctggtgaagttgactcttttgaagcaatcagattttcatcttaaggaaagtttgagaaaccggtttgtttgtttgttttcttcctgtttaggaaattgtgtacttcacaattaccatcactgtaacagttatttggagaccactgcaaaatcactgccaccccaccttaaaaaaaaatgggctgcatgatcacttgctcttcattttgcttttttctttctttttttccaatctgggtaggaaatgggcagtggcgggtgtggaaacgaggcagagtgttcggggggacgactgctttgctctctgaccagctgaaaacctagagtgaattttgggcaagccagctgggacaccaccttctctcggaaagtcccatccccaaatccagaccagtcatcctacgaacaggggtggagtataattctcgcccggaagggtaatttagcacaagctgagacagcagtggcgagggaagggcagtggggggtggggtgcggtgggtgggggcgtctgctttccacaggactcccaggcttcgccgccgatctacaatttgctgaaggagcaaagaacatcctcggctctaagtagggcttttagtgtgctcattgatgagtgaaagtcgccacacatgtcaagctaaaggcagttgttgggttactaacaggacccagcgccttgcaaacatatgcgctaagctgtgtatacagatggcaggcagaataatggagcaggcgccttttataaagctctagctgctgcctgtcttcagacctgggaaatgaaactattcagacttgcggccagatagcgcctgcgattgtttgttaccgttttaatcctattaattaaaacgttaacctgattgggtagaaagcgctgtcccaacaggcgagtcttcttcataataacctactcagagataatgatgtaaaagactcccccgtctgtggcggcggctgtttgatgggtccggaaatctcttgaaggtgaatccaagcaagataaacggtgcggagaggaggcgcggggctgggctcagagcggcggcggcggcggctccactccctccgcgcccaccctcccaccatgcggggccgcggcccatggtgagccccagcagccagcaccatcggctggagacgaagaagaagaagaagaggaggcggcgagcgcgggggaaggcgaaaaagaaaaagaaagaaggggagagggctcccggcagcaccaggaccgacgcgcgcaccagctccggagcccagctcgcgcgcgtctgtggggccgcctgactccggggccgaggcggcggcggcggcagcgggcgcggcggcccgggctgcgcgccggcgcgggaccatggagcgcgggatgcacctcggtgcagcggccgccggcgaggacgacctcttcctgcacaagagcctgagcgcctccacctccaagcgcttggaagcggctttccgctccacgcccccgggcatggacctgtccctggcgccgccgcctcgggaacgcccggcgtcctcctcctcgtcgcccctgggctgcttcgagccggctgaccccgagggggcagggctgctgttgccgccgcctggaggaggcggcggcggcagcgcgggaagtggcggcggcggcggcggcggggtgggtgtccccgggctgctagtaggttcagccggcgttgggggcgaccctagcctaagcagcctgccggccggggccgccctttgcctcaagtacggcgaaagcgcgagccggggctcggtggccgagagcagcggcggcgagcagagccccgacgacgacagcgacggtcgctgcgagctcgtgctgcgggccggagtagccgacccgcgggcctccccgggagcgggaggtggtggcgcgaaggcagccgagggctgctccaatgcccacctccacggcggcgccagcgtccccccggggggcctgggcggcggcggcggcgggggtagcagcagcggtagcagtggcggcggtggcggtagcggtagcggcagcggcggcagcagcagcagcagcagcagcagcagcaagaaatccaaagagcaaaaggcgctgcggcttaacatcaatgcccgagagcgccggcggatgcacgacctgaacgacgcgctggacgagctgcgcgcggtgatcccctacgcgcacagcccctcggtgcgaaagctctccaagatcgccacgctgctgctcgccaagaactacatcctcatgcaggcgcaggccctggaggagatgcggcgcctagtcgcctacctcaaccagggccaggccatctcggctgcctccctgcccagctcggcggctgcagcggcagcagctgctgccctgcacccggcgctcggcgcctacgagcaggcagccggctacccgttcagcgccggactgcccccggctgcctcctgcccggagaagtgcgccctgtttaacagcgtctcctccagcctctgcaaacagtgcacggagaagccttaa

SEQ ID NO: 2 - DNA, 4000 bp, Homo sapiens
ggcctcagccagcagagcccagatgccttctgcagttaagatccctggactcagaatcagaaagctgttaagcaggaaggagtgcgctgccatgaagaggcagacagaagccagagccagtgtgtctggaatgcatcaggtagatgaatgggaagatggctgggatggagttggagggaggagggaagtcagcagccaggggccaggacattcatggccttaaaaagtatcctacaaacaagaagccaggttagctcacctatgaagagggacagtcttaccagatcatgtgttagagtccccagatcctggggagcgtgagaaaagtgcagactcagctggctctagtactagattaaggaggtcctaggtgggcaaggccagctgcatttttcataaaatgccctagaaacctctgcagtttaccaaagtgaatagctcctttggacttaaccatctgcaaggctcattccagttagagtgttccatcaccctaaatgctgggaaaccaagcgaatctcctcccacttgcaagcttccaacagtggcttccaacagtgccactgcagtatcagaaactgcagggaaggtgccagggctgacttccatgaagaaataggagaacaggcaggcagacattggggaggcccacagaatgtcgtgatcagaattcataaagaggctggcaggatacaaatcaatcaaataaacgttagttcaaaaaaattcactacacctgtgagtgagagaaagtcatcagcactgtctctaaaaatgagcctagggcttctggtgacatccaatcggtgggttatcaggagtgccccaggtgatcaggagttggcctcgactcagtcctttttgtgctgtctcctcctctttcccagagttcctctctctcttctcccactaggcagggatgagcaagaggaatggctcacccttgagagctggggtccatagcccaggtcagttctccagctctcccacttaccagccaagacaggaggtgaggattgagatgggatgaacccagcaggcggccatgggttaaaggtcgccatgaatgtaatgtgcccagcacagtgcctgctaaaaggcaacactcccttcctggtctgaagaccaaacaagcagactgtactcaggaaagccagaagaaccttccagctgtctggaccagaaggtgccagcccaggggctgaagaagacgtaatgcccagagcaaaaagcgcctgcagccccctgaagggctgggtgctctggaatagatgagggggcgaaatggggctggggaccagggacggacagggtgggtccagcacctgcctcgcttccgaagggctgctccaacactgaaaaacacccaaccagcttcctttcagaaagactggaatattccaaaacttctcactggaggctccggaggaggtgggctccagctgaaaaggaaatgtggaggcgtgggcgctcccggcctgcatcctgcacctcttacactttggttttcccacagactcctgaagaataggtcagaagaaagggttaaagccttaaaaggggaacaaccattgcggggctcagggaggaggataatgttctttgggctgccgcaccctgatccccggggtcccgaaccctcccgtccctggccaggcctgccagccacagggtgagggcccccttccgccgcaacctgccactctcacaccaatgcgggaccgccttctcttccttccccaccccccaccccaccctgccgtcctttctcccccaatctccgcctctgattggctgagcccccggctccccgctccccctctcctccatccccggtgaaaactgcgggctccgagctgggtgcagcaaccggaggcggcggcgcgtctggaggaggctgcagcagcggaagaccccagtccaggtgggaactggagccggtgggacctggggctcggggaccgccgtcaggcgcccatgcaagacttcccaacactaggcttcgggccacggtccgagggcgcccagggaagaagggcgcagagcttagggaggggcctgctttccaggcaggggcgggagggggatgcttctgcagggcaggggccgcgtggcaccctgatgtctttcggggaaggcgctcccgggctttcgcccgctgggggactggtgtctggggctggggcgctggagaacagggaggaagggcaccaaggacagcctgtgggtctacattccacccagacgtccccaaacccagctcgcagaggcggggaggaggacggatgaaactgcggggagaggatggaggatggcgagctagagggaatctgccgggtgacctcgcggcgggctgggtgcggggcaccggaggagaaggaagccgcagtgccgcaggcggggactgggtggaaggcgggcggacgggggaggggagagctggaaaaggatgagagagggggaagggggactcatttgggaaaggagaggattggaatacggaaatggattaaggatgaggcccgccgggggcttgagagggaggaagagcagaccttctctgggtctggagccgcctgaggacacagaccagaggaaatgaatacagactgcacctccccagccgctctccacccctcccctggctcttctaccctctccagccccagacccatttcttccctttcttgctctggccattgctcccccttcccctcctagatcccaagcccgcacaacatctcaaacaagagtcctcgattcaaaagccagatgccgaccccccttcctcctggatctggctcagggcagcagctccaccccgggacagagagagcattgattgtagctgcagccgccgcgggatcctagcctcacccgtcaaggggctgagcgccagggaccctgaactcgtctagtggtgcgccctgcgcacccgggcgcactcaaccgaggcaatgccctgcgcgctctcgcgggtgcacgccccttctgtggcctctcctgggcgagcactgctctgcagataggctagactaccggctccgcgtcgcctcgccaagggttggttcagccaaggctgcaaaaaacaaaaaaagaccaggcagacagcctatccagggtggctattgaaactgggctggaaaactgcagtcccaggaactccagagagctggacattgggaagcatccttggctcacatacaatcggagatcactatgtctttctctcctccaggaacacgattagcttgtgtcctatccagataggaatagatgctccctatctgggagcatccttagctatggtgaatggtatctagccatccactggggatggcgagtgacttagggatttgtgtctcacgtatatgaagcagtcatcgccagatgttggttgtttttcttaacccccatcataacccggtgggtatgtaagattcagagagattcattcattcattcacaataaatatctttggagtgtatgctatatgccagtaatctgcaaacggaaacggttttgagcattggggattttcttctgaacaggaaatgggaagtccctaaatggggagtctttgtttaacagatacagagttttactttgaaagacaaaaagagttccggagatgggctgcatagcaacgtgaatgtatccagcactgctgaatatactgaatttaagtactgaatttaaatggttaaaatagtaattattatgctttttgtattttaccacgattaaattttttttttaaatacgaagcctcagccctcataggtcttatattaccatacactatgttaatgtaagaagaggagaaagagtggtaaagttacttaaagtcacccagctagtaagtgctccatggccaagcgcagaaacacaccgtgactgggcttgttctccctccttccttgctttccctgagcaggaaagagccagtggcagtatcatgttcagtgagatgcagggacgagagggggaatggagaga

SEQ ID NO: 3 - DNA, 4000 bp, Homo sapiens
attctaaaaggaaaacgcagaagccctgtctttctgaggcttgtctgcaacatacgctcattccttccaaattatttgctggaaaaaatttaataaataatcatagagtaattaacatgttccagttcctgtctatactggttgatactgattcaacgagtatgaatgaacttatgaggtgggtgacgttgttatccccagtttacagatgaggaaactgaggcacggtttaacttacccgaggtcatagcagtagagttaagatttgaaatcaaatgtcttactctctctcatcaatgaaaactgagctacgatctatcagctcagcacataacaacacaggatcatcctaattatttccaatgtcccccagagtgattcttttttcttatgataaaaattatctggaaatttctaggcacataagcagctgaaaaggttgcatgtgaggcaatgaatagcagaaatatttgtgtgccatttttatatcaacatgttaatgtgtgctaatgaattttagagtggatttttttaaaaacatgactattgtaattaaaagcttatgtgatttaaatacaagatgcaatgatgattaccagattctattcctctttatattttacataagacttccagggttccataagtataatcttgaaacataggacattcctggaaaaaaaaattgcttaaaactatttcagtgtgcaatccacctctttgtaaatgttactttcttccatccaaatattacatttggcaacaaaactctccgctgagagctttctcttccttttgtgtcattgttccctaaataaagcaacacatgaaattcctgacggcaaaaatcagactcagatcccaaaacctctgtctttatgcaagatttatcttttgcattggaaacggccaaggaatatgaagaggggaaagaagaggcaaacagacaagcatgcaggctctgaggaataaatgcccctcaggacgctgtctcctggggaattgcaaacctcagtccgtttctgaggaagtgcggtctctgcatttctgaaagaggtatttcccccccttgacacaaggagcatggtaatgaattgactagttaaaaactgttggttggaaaaacccgtccctgtgtctttctgagcagggcgagctgagctgtccgcgaggctgcggcaggaggcctcgtcctcccgggcagggtccctcctggaggctcccccggtctctcccagacgcacccgcgccgcgtccttgttccccgggagcagcctccctccagccgccggtcctgggagcttcaccgtccaaacgggagctgagtttgcaagcggccaggcggcggtgcggctggtgctgctgctgatgtcagagccagaaagcagttgtgattggatctaattagacgctgctgcagcaaatagacaagctccctgcgtgattggcttcaaagtggctggtgccaaacaactagcagaggcgcaaaagtagcctccctgcgctgggagcccagagcaggaggcagagcccgcgggaagctcggagcactcaggacgccgcgcgcccttccccgccctccctgaccagggagcagctcgctccaggcgcccagccgaggcccccagcccagtgggagcaagtcatagagaacaattcgagagacagagagacggagcgcgctttcctgctcagtcctgaaaagtgagccgctcccgggtttgcaacctcaagcttcgcagcagcggcggcggcggctgccgggaaggaggcaggtgcaggtgcaggagggaggcggctctgggctccgcgcctgggtctcggccatggcctcggtcctggggagcggcagagggtctggagggctgagcagtcaactcaaatgcaagtccaagaggaggaggaggcggaggtccaagcggaaaggtaaggaccgcgtggcgcgccggcccctgccccccttcacccccggcttctccaccccggcctctcatggggtctccgggcttgtccgttgtgagcagcttcactttggggtgctggcgggatggctgctccgtgcagggcgctcgggagttcagatcccgtggaaatgtctggggcctcctcttgcccagaggggacagtgagcagccacgctgcgacatgtttgagggacccggacgaagtggggcgagggcggcgaggagctccccggggaccccgcgcgtctccgggccccgcagtccccagtggccggccgggctggcactgccttccaccctccggaggccatctcgtctcccagtgccaaaggaattacccaaaaacgggggaacgagccctcgcgccagctactcccatccaaactgtcccggaggaagggataggcgaagccctgcgatcgcctctccaaattggctggcagtttttactcaatgtggtgcccgtcgatttgtaaacattgggtcgtaaagagaacacagggctcgtccttggagaaataagcagaaatgaatacaggaaaacagaaagaagcatcatattttgttagtggtagaaaaaaaccgcaaaccaggaaagcaggaaaagcagccggctgacagcggccactgacaaactcagctgtgccttgttactgatattcctggggctgggccgcgctgaagttagtcaatgctacagcaagggagggctttcacactggggattttgcaaaattagcaatcgctccaatatgagagcaatgcccccagtgccatcgtagcctgtgtgcatgccaggaagaattaaaagattcttctcatgccgacccttctctcctagaggaacctgtgttattgtcagttcctagtgagcctgcaggagaaagttcagttctaatcatgatttgaaatgtgctgattttttttaagtgaggtagaagtataaagaacggttggaaaaacacagctagaattgatcagctttgccagttgtttgaaagcaggaggcaacgttaggtgtgtttggggttgtccatctttcctgaagaattttcatctttgcattggcctaagataagtttctaccagaccgtttcctgtgtgccctcgaaccgtcaccaggtcctttattgcctcttccaataatagaaattatccagacagtcagcaggcataaatgtcaatagcaaacagtcattcattatgaccgaacgtcaggaccactgggagggattggcccccacaacttcctcaaaaggttttggagcctttggtttcagaagggaggtgatgttgtggttctcatttacctctcagctgctaagtgtgcgcttgcgattcactttgttgtttgaaattatcattttgaaacagacctgttagtgtcctccaaagataatgccaacacaaagtggcattgatattgagaaagtcaccggattgaataatgaatatgacttttaaaagaggaaaaaggaagcatcatctttacacttgaaatgttcacatttcccaatattttttgattagtctatttaaatatttagagttgaagaatgtggagtaatagttcgcaataatgcattttataaatataaacaggaggaaagtgttgcctttctccaaattcacttgccttgccaggaagcgtcagtcatgctagcttagaaagtattcaatttagggggaaaaaggaaatctggggaaagacttcatttgctataaacttaactttagcaattcaaaataaaactcctatagcaaatatttccataccttggttattttgaatatgtcaagtcccttaattttcatagccaaaaattgaagcgggaaagggcattcaggttttgtacactgatttctgttacgaagagatttctggcgtgcgggagaatttcccagggcacctgccggcagctatcttgataggaaagtcaaatcaaacggctaaagattcaatttttggggaaacgttaaccatgtagatgtaactgatcaaattaaaaggtaaagtaaccagctaagagacacat

SEQ ID NO: 4 - DNA, 4000 bp, Homo sapiens
cgtgaatatattactttcataaaaatgtaaaaagaaaaagaggagtcagagaaagaaaatgaattgtcagaaaaatttagaagttttatcaactgaaatgcagaaaagataaattgtgcttgcatttcatttttgttgttcattccaaacatttatggattagactagctgaaatgaagtaattaagagactcaatagaaaacattgccaagaataaaaaataatttgaggaaaccatgaaaagtttacaggttactctgtcacaaaatactttgttaattcactaccccgcagcaacacacatcaccaaggctggcttctggaatgctttctacttgtagccatttttgaacaataggtgattccgcttttaacaacactgttagaatataatgtagcgagttttaccagagatgtttaagactacctggcacaagtaaatttcattgtatacatgtatatacacgagggagggtgatcatagtctagaaaaaaacaggtcttcagaagtctagaactttaataaccttaaatccaaattattccctgcgtccatccataatgagaaggaagaaatctacacttgcatttcttccacctttcacatctttctcatttaaatcctactgtacttgatttgtgttgttcccaacgtactaggtgctatgcatgacgtagaaacgtgtttccttatatgtatgtactagcaggctccttcaagcacatgcctaaggttgaaagattcaaatataattatagcctcttaaattattgcgtcagagcccgccctatcccctcagaaaaagcccccttttacaccatcaaatgaaatatcaggttatttgcactggatattttttaaaagaaaatatttgattttaaaatcaaagagttcttggttttccatcatttcactaattgtcttactagagacccgagtctcctttgtcaaaatatatttcagtacgcattttaaaaaatatgtgtgtgtgtatacttaaatatatatatatataaagtcttggacttattttcacctagcctggggcatatcgtggatagtttcaatcgacaaaacaggcactctctggcctaggagtggaatccatcctcaattttcgcaggctcctcacaattctctatttggaagaagtgtccctctccttcccttttcttttcctcctttactcagcgtcagtccccgcagccatctcctccgaccctttttgtctacgtcccagcgtcgcgaaccacagcggcggaggtggagcggggagaggcgttaggccgggcggctaaaacgcgccgttaaagtgggggagagattgcgcggagcccacgcgatccctgggacgccggagacaacggggctcttgggaaggcgcggagcccggggaagccggggatgtgcgcgtgagccgtgcccgcagggtctccccgcctccgccacctttcttgggtggctctccgcctcgtcctccctccgagggccgttggtacattcctagtgactccaagcgcttaaaaggggcccgggaggatgaaccccacagatctgaacctgatttgtgtgtgcaccgcgtctccagcgatcccggatccactgcgctgccaggggcctgggggtgggtctcttgctgtctctgcgacgacatccttacgtttcggcactctaatgctgggtttgtgcgtgtgtgtctgcttagcggtctagcgggctgttaggctccctcgcccccagctccttggctcgctcagctcctccaccgcagcccagcagtgagacgcgcgcgcagccagctccccacgagatggaacagaccgaagtgctgaagccacggaccctggctgatctgatccgcatcctgcaccagctctttgccggcgatgaggtcaatgtagaggaggtgcaggccatcatggaagcctacgagagcgaccccaccgagtgggcaatgtacgccaagttcgaccagtacaggtgagcgcgctgcagcttcaatgccaggcggcgcccactcgccccgtctgaggaggaatggacgtgggggacgcagcccaaagtgactggctcgggaagctcgggccgcgctgcgtccgccgctcgccccctcgctggccagccgcggggctggcacgactcgcttggggctccgcggccacagcgcaggcggaaggtggatcctactggccttgctgacctccggccgggaacggcggacaggcgccgggaagggaggccaccgcgcgtctgcgagattttctgttctcttctctcccgcaaacccctctgcttctaaaccaccagtcctcctgcccctggcctcgggagcaatgcccacactcccaagccatcgttaaccccgggcgcggagatgcggagagaccgcactcaggttcgggccctcctgacaccttaaggaaccgtctggccggactagcagagggtgctcccaggggagcactacatcagccatcgggagaagtgtgtgatgttgaagaagacaagtcacccgcgtcagttctccatcactgcgccttcggtcgcctgcaaccgggcaccttatagcaagcatttttactcatgtaaaatagcgtcttgtggccgtcagctgccactacggaatttctgctgttccctttcccaaaccaatttaactaacttccccgactgtgggtttattcaaatccactgccaagtttcgcagattaaatattcgaccgtcgtttttttcagcccccaaatgatctgatttatcttatccttgcttctgacgatctgtaatgtaaattaaagacccctacttcccagatgtacttgagtgaggtgccctggtaagctggcttttttgcagccccggcttggtgattaagtcgaatctctctaccaatcctccggggccagaggtaaaatttaatcaccccgaagtgtgagaggttctactttttctgagcagttagtgcgtcagtctttgtggttttttgggtttagggttaggagaaaggggtaagtgaaagaaaagaataaggaaagaagtaagtttgtttttcttgggagcaggttcttttagtcactcttcaacatgtgggatgtttcgtaaagttttgttggcatgggcggtttcaactgtattttaggatttgaaatagaaaaagtgaagaccactaaggatcccatttttcatatacaagtgacttgaggaaattcctttggctcctatcagcttagttcatggtagagcccttctgtagccgtgaaagctagcagagagtctagcttttaaattttcttgcatttgctccaggtaattgaagacttgttatgggacaggtactcttccagacacttgacacatatgaggaatggcaggcaatgaagaagttgaatgacttgcactaggtcttctatcgatagcggctccaggctcccggggttagcattgttgttccagagcctacactctaaaccactgttaaaccaggacaggttgtaacagtttttaatctttaatctttagaacaagtgtattttcaaggaccttgaactagtctcgattgacaaactctaaagcttttgaagtgcaaccagctgggttgatcggtcttttcacagatatctgaggtacagctcattaacataatggatgtagtcccgagggggcagttgggggaagacaggagatgggagagaagtcaattctacagtattttttgcattaaataggtgcctagcgctgtgaaggattctgttctctgactttgggagggccagtgcagaagaatcaagacagaatatgctcccgtgtgggccaggctgtgaattctttgaaagaagctgcagagaagcaacaaagattatcctaagacttctggaggaagaattaggatccttctgcaggaactcagtttactgtgaattgaaggttgtgtacacagcttcttgttaggtcataaaggctacaaagtagggaaaactgaggctaaaaagcacttactaagt

SEQ ID NO: 5 - DNA, 4000 bp, Homo sapiens
gaggctgccctgaaaaagcaaacatgagagaggacggggtgcaggtaaatatcattaacgtgaaaatctgctaccccagccaagttcaccaccagtattcacccctacaggcggggccgctcggaccctgctcccggctccgcgcctgccactccctttcccgcgcagccgagatgccagccccagtgggcctggcggggagtccggcggggtccggaccgggcggctcgacccccggtccccacggcaggaacgactcagcctcgcacctcgggagctgtaggtgccgaaaacgaaacccgcgggggcagcgcacgccgcgcgagtctcggtccggcggcaacccagatagcgattcaggggctttattcttttgatggtgattaaaaaaatatattctatttgaacccgtaaagcagacgagggcaaatcaagccatcccccgcgctggctcaccggccaccgcgcccagcgccttcctccccctccggcgggcgagcgggcaggggcgcccgactcctaccttcctcccgccagccaccgggggaccagccgcgctctccggggcgggggaggccgcccgggacggggacccccaccttccgccttcggaagcgggttggggcgggggtcggaccccgagtctctactccccgtccctctgccccccggcgcggcccgacagctcccagccccatcctggcaggtggcttgggtggcggtagatgccgggcgggaggaagatgtggggctgctctggcaggttgggggtgcgaggaggaaaaaaaaacagagaaagacacacacagagagacagggagagagcgcgcgcgagagagctcttgtctatagatttatccacataatatatatttatgtagctttttttctctcgacactgatgaatgcgcgctcggatccccgggcggactccctccaagccggctcgcttttctagtctaaataaataaataaagccagatggaagaaaaaagcgcccattccacctccgccgccgccccgcccgccatccctgcctttgcttcgcccgcctggcgccctaatagagcatagcttggtggataaagcccccctacatacccacacgaaaataaaaatcactatttttaaaatacaaaaagttgcacctgctgctattacaaaaagaacccccaaaaggcaaagagaggaggccggctgcccggctcctcacggacacccgctccccgcggccgccgggcccggaatctcagcgcctcccgaagagccatgcgcctggcgctatttatagccgggggccgtctcggactgtaccatcgccacggcgcggggccgccgacgggggaggcgcggtggccgccgccccacgccgccctgcccccggccgccgcccgccgtggcgcgggcccccacagcgcgcccattcccggccccccgcgccctcctccgcgcgcgcacactcgccacccccacccctggtctggctgggaacttgaaccggtccagcctgtttaaacggaaaggacagagatcctgtctgttcaatgtaaaaaaaaaaaaaaaaaaaaaaaaaagaaaaaaagaaaaaaaaaatcagatcagaccgagagagagaggagagagggagagagagagggagagagagagggagagagagaggagagggagggagggagagagagaggggggagagcagagagagagcgcgagcgcgagcgagcgagagaagaggagaaagagagagagcagagagcgagcggagagcgaggtgtagagaaaccgagggggagagaacccgagtgtgtgtatgcgtgtgcgtgtgtgagcgcgagcgagcgagagagaggagcgagagagtgtgagcgagaaagaataaaaggaaagaagattttctctatgtatataaagatggccacgttagcaaacggacaggctgacaacgcaagcctcagtaccaacgggctcggcagcagcccgggcagtgccgggcacatgaacggattaagccacagcccggggaacccgtcgaccattcccatgaaggaccacgatgccatcaagctgttcattgggcagatcccccgcaacctggatgagaaggacctcaagcccctcttcgaggagtttggcaaaatctacgagcttacggttctgaaggacaggttcacaggcatgcacaaaggtgagtacacctttccctcccaactttgccggggagcaggagcgggctggcgggccgaccggccggccggcgactgacgagcggcggactaagcgagaggaagcctcgggcgggcgcggtggagggaggcgctcgggcagcggagaccagagctggggtgcgtggggagctgttcgctggggcaagactgggttttgggcgaggtgctgataggaacgatgccatggagagagcagcgggcgccgatgaagagaaagagagaggggatcgaggagacggggcttggatttttgggtacagcgacctgaaagatggggatggggaaggctgcaccggtcgagcccaggacgctgagcggacggactcgcgggctcctggccggccgaggaccgagggtgctgtccatcgccgtggtgctgaaaatactaaaggaggtggtctcctcatcctttgctccgggctagagtagcaggagcgcagccgtctaaaagggagagaggtgacaaattcaaagagaaatttttatttaaatgtaacagtaaactctccctgtcgagctgtgtgcctcaataatctgattgtggtgtgaatggtggtgtgtgttgggggtgggggggttggatgtttgaaggaaccagtgataaaacctaaggcaagaattagcaaggaaccagccatcccctgggtggagtggggggtctggcaagcctggatagtccccttcccaggaaagcggggctttgggaaaaaaatatgtgtgtgcgagatttgcattttgaaaggtgtaccctaatttatcccaaactcaccatgcagagagctttatagtacattatttctcccttgaagcgatcattgccagtgagtgcttgggggagggggagacagaataatcaaagaattaaaacacagcaactttttaggaaagtggtcatgggaattgtccgcagcctgcctgttttctccttgttttattatctttaaagcagagccccaaacgtgttcagttgtagaatgtgtgtgggtggctggtgggtgacgaaattagcccagtgctccgcttcctaacagtaatatataggatgtgcagcgggaatgaatcggtgctggatctatgtgggcaagttaaatgctttctgagagagattgatcgccaggcagggaaggagcacggggctaaggaagttgtaggggatgtgtatggatgttccgtttttaataaacagtagtgtggagagccgccgaagatgctgttacagctggtggttttaaagatgaaaacacacgcacacccacccccacatagagagcagcctcatccttggccacaaatgggctatggacacagctgatcctccagcacattaggtgcagagcgcagagctgtctggctctctaagcagcagcgattttcactatcacaaccaccctctttctccagccctcccttcgttcgaatactaaacagagctccaaactcttcatagttggagtcccagagagcagtttttattggctttagtatcttccagcttgcctgctgaggagtaaatcttaaagttaatggcatgttgagtaacacaaaaacacagcagaatggaaatatactgggtttgttggggtggggtgagggtgggggctgtaatggagagagaaggcaacctttatccaatatggagaaaatgtctgtctgttcaaaagagagattggaaaggtggaacggggaggcagccttcaaaataatattcgaagaaaaaaagaaaacactttctttttccccccctccctctcaagtcaaccatatctttgtagtttttc

SEQ ID NO: 6 - DNA, 4000 bp, Homo sapiens
tcacttaaaatcctagaaggaccttatatatagtgcatatatataacacacatatacacacacttaagtggtttattttctgccttccccatttaaaacataaattccttgacaataatgactgtgtgtgtgtgtgtgtgtgtgtgtgtaatttattgtcttattcgggttcctacattaatttgcattaatttaattaataaatgctctagctctaccatacaacccttttccttctttctttttatcaacaccatcgccatgagaagagcaaaaacaagtgtgcctgtattttgagggttctcatagtcatcaacattgaaaatgacaagataagaaatgtcaagataagaaaatgacaaaatttgcttatcttcaagaccacctcctatacacagaatgcagaaaaatgccccacacctcgtggaactcagtaaatattagttgcattgaattaacttcaattcaagaccccattctacagtttataaagtcaaaagttgctcttagtaacacgctcagtaatatgtgctgtgttttgaaaatagaaaatatcccttttcctcaaatccatagatagtcatattaagcgcaaggacttctgtttatttataatgattctcatatacagatgcatacaactgaaggaaggatggtatgtgtttccagaaatatttgctttatgatgagatatgagtgaagttcctatttttttcttcctttgagaattatgtttttattatcatttaccctagtgctcattttcatcctcttcaacagaaatttagcagggagactggttgaaaaactattcatataagttcctccggaggcttaatcatcagtacattgtcttggaaccactctggtgttttctaaattaaatatctctgtctacaacaaatgcgaaaagtacagaatgtttccgtactccttctacatcaaaattgcctcctacaggaacgagaaaatgcgtgtcaatgtgaattaccgtctacaacagctactctccaggctgatctggggtcttgcacacaaagggcgaagagaggggcgtggggaggctggaaagcatggttgccccgcctggcccggcgacgcccgctcagcagcctgctgaggagtggggacgaagagcagcctaaacttagggctcgggatatttcgatgccacccaaattgccgtcctaccccaacgaggcagggaaaggagcggagcgcgcgcgcgagctgagtgagtgcttacgtcgcagcgagatctgtgctgggataattagagaggagttgggctgagccgagtcctctttcagcagcagcagccggagccgccgccgcagcccggtggggcaaccctgactcggaccgctcgggagagccccaggagaggccagcgccgcgcagcagccgccccgctgcgcccacctccccggctgctcccggagggctcacaaaggcggtggccgcccgagtggccttctccatccaggcgttcgcgtcctcctccccaccttctctcccgaaggcgaaaatggcagggccaggcgagaacctgggacagcggtggccctagccctgcgatcctcacccctcctgctaggagaggctgcgggctgcccgcggacgatgtggccgcggctgctcccgagcgcatcttcggcccgggtccccgccgccacccctcttctctgctccttccatcccgcccagaggagttgatgccgctgtcgccgccgccgccgctgctgaagccgcggctgatggatgccagggagtgccgcattgcttagcgaccccgcctctgggtttgctggtaggagcggctgctctttcttctttcttgctttggggttttatagaaaagataaggacatttttattttattcttcacaacgtcctccccttctcttcgtttttgaaatgtgcattcccagagatatccccggtcccctccctccccctccccccttttctccaaccccgcggcaagtccgtggaaatgaagggctagaggaaggcagaagttgggggtggggttgggggagcccacgctggtaccaacgccaccagaacccctgctggtgccttatgagatcacggtgtatctcagaggggtggtgggaaggtgcgctatctgcagagtcttcacctaattggatcacaataatcttaaataaatcacacaaatttgtcttttaaaaatagcgtctttgaataagtacagggagaaataatctcctttctcccccctctttctctctgtctctttttctttctggcaaagatgatctctctccgccctggagctcagcgctgaagagctaccttattattaatcagaatttccatcgccacccctggcaggcgtatccttcagcagggaccgcaggaacattcacagtgcaggggctgagatgtgcgtgggggttgtttttgttacatcttggaagagaagagaagaggacagtaccaagatcagaaacacccgtgctaggtggaattaggggtgatttgttaggaaagagaaaggacaagaagaggagtgcggagcccttcaggggttcacatctctttaaaggaaaggaaagagggagccaaagtagggtgttgtattttagggggcagaggaagaagtttacaccccccggcccccccagctttgctgggggaaagcaggagcaacagggcacttgattggacaccaagattattaatttcctgtaggggagaggaagcaggcagcaggaggtctgggggctggagtctggtggtggcaaggaccaggtttgctttgggacagtcaacaaggtcttctgagggaaagctcagagataggcagaacaatgactcatttgcaagccggtctctcccctgagaccctggagaaagctcgcctggagctcaatgaaaacccagacacgctgcaccaggacatccaggaggtgagggatatggtcatcaccaggccggacattggctttctgcgcacggatgatgccttcatcttacgcttcttgcgggctaggaagtttcatcactttgaggccttccgcctcctggcgcagtactttgagtaccggcagcagaacctggacatgttcaaaagctttaaggccaccgaccctggcatcaagcaggcactgaaggatggcttccctgggggcctggccaatctggaccactatggcaggaagattctagtcctttttgctgccaattgggatcagagcaggtaaatcctaaatccaaacttgtattctccttttactctcccattttccagaatttaccccgagtagtgtcatggttttgtagatttgatatttttgtttatttggcttggagaaaagagaaacaaaccaggagatgagtttttggtgggcaccctgggaagggaggagggcttgtatttttacttttaaaacttacttcactaacacccactttctactgcagctttaaggtgctaccttaaccacgttattgcacagagatctaaatcacttaacttgtaaataaagcttctctgtatgtttcaccttctgaaaaagtttattgggctggataaaccagtaagaaaatggggacaacttttcctccttcttcctaaaaaaattcttaaactagacccatcatcattgtcatcatcatcatcatcatcctctctttggtactgacgttttatcttttaagcatagcctggcgttcgaccaaaagcaagtagttttgttgcttgggaagttctctgtttggtgatgtgtagaagaaggaataatatgatttgtgtcccttcagtgaaaggaagagttgcatcctctgtcgctgagcatgcctgctgacactgaaaatgtacactgactggtgtatgtgtcctacacctgccactaatctaaagaatctgtctcctgtctcatgtgatttttcatcttttggaaggaagtggaaaatattcagatgtgtcagttggtggactttttgagctcatgtgctacttaatagaga

SEQ ID NO: 7 - DNA, 4000 bp, Homo sapiens
tgtcgcccccagcttccgggatgcaggcccgccggggtctagaggggcggctgccgtgcgtccagcctgtgcgcaggcctttcgccgctcggcgccccaggcagcctcagtttcctttcctctgtttgcgccccagtgaacctccgcacctctcattcagggaagagaattccccgcgcagccgcgctcgtttcttcctctgggattttcctgagaatccccaggagttggccacgatcccatggggggtttccttctacccagccccgcgtcctggcctcgtccttaacccccgggttgccttcactcaggctgggaatccacgattgatttcctactacggaagcgggtggcgttcccagcctgctttcggagcagcacgggtttcgtgcagggtgttatcccgaccccttcccccatccctctaatctggcttgagaagcccgtgctggagagaaaaacgcggccttaaaaaaaaaaaaaagtttaaccgaaagcgtgagagccacccgccggctgttatctggggctgaaggctgcggtaatcgatgggttatttttacgcggtaatagggccctgtgattgctctattaacctttagacctgtctgagggactctccggctcgcagccccgctgcgctggggcctccaggctctgacgccgactcccaactcaggcctgacacattcccctcccccataccctggaagagccccctccatgaagaagctcccctggaccgcctggctccccagcccttgccacgtcccttggattggtgcagagccgccgcaggctgcagaaaaaagggggaaagattagaagagaggaggccacaggagatgggaagtgtcgccaggaagggatgcagattgcataaatacataaaattgaggctgaggcctgggctcccgaccatctccctgggattttgggaaggcaaaagggaggcttcggtctctacgctctgattttaggaggcagtctgggtgtctcctgaacctccaaggaatccggggctgggaggatccccactacccctgcccaggaactagcatccagccgggcaccccgggtgacccagtgccccacacaagatcgagagttgagcccaagaggtcaccttcttctctactggccccgcccctcgcccgccgctgcgggatgaggaccacaggaagggggggcggggagggagaaagggaactcattaataaagctgaccctgggcaccacagcgaacccaatcgacctccggctgggttgcgggtgattccccgctccctggcggtagcacttgggcattttccgcggagaccccagagcctggactttgcctgctgggggagctttccgcacagtcccgcagcctgcgcccagcggaggtgtagccggggccgcgcacccccgccccgcccttgcacgtgactcccacaggccagtcagcgccctagggccgagttgctgggccggggacccgagccgcgagctggggacttggaggcggccggcgcaggggccgcgagaggcttcgtcgccgctgcagctccgggggctcccaggggagcgtgcgcggaacctccaggcccagcaggtagggcttttttcttccctttctttgctccttcccgcggtcccccaaactcggagcttctccgcctttgcttgtctggaggtagagaggtagctagtgggaggaaaagagacgtgcgctactcacttcaccgaaattgcccaacccctgctctgcttttgactttgccttagcaacttctttaagtcaaagtaagacttgggggcaaaacagagaaatattggaagcgcctttggattctttccgtgtgaacttgaacgctttcaatccctgtccccgtgtgcacattctccaacccttgtttgcatatcgcaggccggggcctgggtggtgatggtggccgcgtgaagttaccgggactgacgggcccgggacaggctgcacggcagctcgcacatggagggaagtagacggaggcttgtcgcccaccagcgactccggggacgcagggtggcagtgccaggcagctccgctgggcctcaggggcccccgggagccgctctgaggtgcggagaggctgctgagtggcggaactattcatgccctttctggccggcctcctcgccctcggggctggggtccagggactgaatgctcctctggaagctcaccaccccacctgcccgcgctgcttctacctgaaactggccaagggcccgagcccggaccggagccgtgacttccctccgccggccacggggctgcccggatccgccgggttatgtcgcttggctttgggctcaggggtcaccgtgggcagaggggggtgccggggtcgcggactgccaccaggttgaggaaaggaggggccttttggctggggaaagagcgtggtgggggacccgcggccgatggaatccctggggcagcgcggcccgcaccgtggaggttggggaagcgcctcggggaagtgtttcctgtgttcccagaaaaggaagacaaccgagagcaggtttcaggcttttaaagaaagcctggggtgtggaggtgatgctccgcacacgtctgtgtctcctcccctgctgcggccggcttggttgtgccggctagcgtgcgaccgtcctcctcgctgcaggccgagagcggaggcgtaaacccaggccagcgaggagtgtcctataaagggacggggacttttcggcgcttgcaattctcccattctgaaaaatagatcggaagagggctattggttgattcttgaaaggggagcgcatttcctgttggcctgcgaatttggggtgaactgggacaagtgatcagaaggagagcaaaaactccccgattttggcagcctcgggagctgctgggctttctccgccaactgcaggatccaggctcaatttcaacaaccagccagaggcgttttccaagagcagctaattccttgtttttccagaaagttatagaggagtattttctccaccttctgttgttctagtaatccaactcaggcactatatcagccatttgaaaaggcagagaatgtgataaagacaaatattagattgatgacattttttgcatttaccttttaaagtctgcaagttactacctgtgtgtatactggaagttggattataaaattctaaatctcctttcttttccaaagttatgaaagaaaaaaaattacattatcttgaagaactgcaggagttgagtattccagaaaatgcaatgaaataggtcagctacttgattttaaaagtcaaatactggatcttttattaaggtaaacccataattctttaactttattttcaaagggaaaagttggtgacctcaggtcaatttttaaaaaaatctattctctaaccaaacttgctggaatgaactatttgccaaaccaataagttattgcatattttgaaagcaaataagcttttaggagttaccatgtgactatataatacaatacagtactattccattattattactagtgatgttgcaaaaaatggtgaaaagcattatgtagtgtgtattaaagattccatttccagatttttacagtaataaagatgatcatttattatagtatatacatttgaggtactttcttgtattatactagaaatctgtagtaatagtcaactgttatttagaactttctttttgcctgttaggacagttttataaaaatctgttataagtgttttacaaatattaatttataatcctcactcctaagcttcacgatgactctacaaaataagtacctttaatatctgcattttgcagatgaggaaactaaggcacagagaggctaagtaatttgtctaaaggtgtttattccgtaagtctcagagcctggattcatatatagttaacattcttgtaaatctactattgaaataaaaaagaaaactttgtcgggagtagttgcctcttcttaaagagagaaat

SEQ ID NO: 8 - DNA, 3428 bp, Homo sapiens
agtttccttccaattaacggagtggcggcgaccttttaatttacccccaacgggtgagaaataaacttccccaacgtggccaggcccaggaatgggactggagtcgatgcccttttacccctccccgttctaatttccagccctggccttgagctgtggctgcctctctttgggccttgtacctctccgccgagtctccgggccccgtaggtaaccaaggcgaggcccggagtagcagctggaaagggaggaaggagccctgaaaggctcacgcggccccgggacaggccacatcggtgcgggcctcccaggttccggagctgcggggtctcttaggcgaggctgccttttcccaaaccgaacttgccttccattcatgccacttgtagttttttccccagctgggattcacggagcgcaaccaggcttgcagcgctcatggttagagcctctgaggctggagcacagggctgggtcgccagccgcctgcgcctgggaatcctgattgccagctgatgagaaaggcgggctgggcgcgcgtgtgcgtggggtcgagggccggggaccgagcgcgccgcacaaccaaccaggccctcaaaaccttcgccctggtggcggctggccgctccctcctggccagctcctccgtggggtcctcgtagcaaaggcgaatttaagggttgcccgggcgcccctcgctccaggcgggtagctgtggggacctacacccgcggtactccctgagcggccggtccctgcctggagtgccctggtagggccggcggcggctccgtttgggacggatcctgcgttgaatttgacttttcgagggcggccgcgggtaaactcgcctctcccggggaccgcagggattatttacagggagctcgccaaccaaacacaacagtctaacctttccaagtcctcgtaaatttttacagctgggagccacggcgaggcaaacgaatctgttggtcgtttccgacttcccgccagcctgtgtggcttctgaaacaataactccttatgaaatatcataaatatagatttaaatacagtagagcgacaatgcgatttggctgcttttttatggcttcaattattgtctaattttatgtgaggggctccgctggccgcactcgcacgcgggacccgcgccttcttgatggcgtgattaattgtgatataaaatagtccgcttaagaagtgtgtgtatggggggggagacgggagagtacagagacaaggctagatttgatcttttaatcgtcgttggccacaattaaaacaaaccccatcgtagagcggcacgatccctttacataaaaacatatggcttttgctataaaaattatgactgcaaaacatcggaccattaatagcgtgcggagtgatttacgcgttattgttctgctggacgggcacgtgacgcgcacggccaatgggggcgcgggcgccggcaacttattaggtgactgtacttcccccccggtgccaccaagttgttacatgaaatctgcagtttcataatttccgtgggtcgggccgggcgggccaggcgctgggcacggtgatggccaccactggggccctgggcaactactacgtggactcgttcctgctgggcgccgacgccgcggatgagctgagcgttggccgctatgcgccggggaccctgggccagcctccccggcaggcggcgacgctggccgagcaccccgacttcagcccgtgcagcttccagtccaaggcgacggtgtttggcgcctcgtggaacccagtgcacgcggcgggcgccaacgctgtacccgctgcggtgtaccaccaccatcaccaccacccctacgtgcacccccaggcgcccgtggcggcggcggcgccggacggcaggtacatgcgctcctggctggagcccacgcccggtgcgctctccttcgcgggcttgccctccagccggccttatggcattaaacctgaaccgctgtcggccagaaggggtgactgtcccacgcttgacactcacactttgtccctgactgactatgcttgtggttctcctccagttgatagagaaaaacaacccagcgaaggcgccttctctgaaaacaatgctgagaatgagagcggcggagacaagccccccatcgatcccagtaagtgtctcctcccttcaaatccgccgccgcctccacgccggcctcccggatctgctggcccgccaggtttctctcgagcctgccttcgtcctcgctggaagcctctcgagttggggccaggagccagaagttggtgtttgggacgcctcagatagggccccaagtctggagagcagtgaagagcggcccgcagggctacgggagaggaggcggctgctgcagcgagagggggcggggcgggcacttcgggacgagccaagactggccgcccctctccttggctgcccaggcccaggaccgagatactttgggccgttcttcgaaagcagtgcagcccagagagccttttgtacaactagattgtccgtgagcggcggcagccagggcagccggagctgggacgctgggggagacggccgattccttccacttcttgccttcggccagtggcggcgtaaatcctgccaagatgaggctgcgggcgacccgggccacaagggtccccatgacagattattcaaataagccacagacgtgatcagcggccttagggcgccctgacggcttgcccagctccgaaggccttccaggaaggttaaataaggagtggggggcgtagagggacaggttgggaaagaaagacgaagtcagtgaacgggacagaggaatcctaatcttgctacagaacacaaggcagcatgctttccctctgcgtggcaaggagacctgtttccaaatttcattctatacagcgttttgagagtgggaggaaggagaagggggacaagaggacagagtaggagaaaggaaggtctcggaggggagggcgagccaaagttttactgcgtgcaattttaagtgactgtctgtgcgtctgtctgccagggttccattgtgtccgaggcctgactgcctttcctaaccagttcagcagagttctgcacttcggccagagaccccatgcaggaggctcatttgccccagcgggatgtgcgtcttctgctcctaaacccagtgtttctcttccccgcagataacccagcagccaactggcttcatgcgcgctccactcggaaaaagcggtgcccctatacaaaacaccagaccctggaactggagaaagagtttctgttcaacatgtacctcaccagggaccgcaggtacgaggtggctcgactgctcaacctcaccgagaggcaggtcaagatctggttccagaaccgcaggatgaaaatgaagaaaatcaacaaagaccgagcaaaagacgagtga

SEQ ID NO: 9 - DNA, 4000 bp, Homo sapiens
taattacgctgaataggatcgtattgagtttgtaataattagcaataccatccctaaggaaacagggtttggtctcactgccaaatcagaagtttgccttgcctcaagagaaatataagtattctggaaaaagtcttgcaagtgtttttgataagaattcaaatctcctcaggccattgaatatcacaggattttgggaaaatgcccagttaaaatcaaggttgtattttaaaattctgttagcaaaagtatttgcaactgaattatctatgtgataaaagttgcataagaagaattctctagaagacgtttggtaacttgcaatcaagtagtttaggtcttgcttatggttaggtgtccctagagatctttaaaggcattaccaactccctctttaaaaaaatcacaaacacaaaggtagagacagtgcattattttgactctcaaattccctttccacttcaacatagtataggctaggctcaattcagcgttaaagttcagtggctttatgtgacaacaacaacgaaagtgttcttttcacttccaaaagaatcagctgtggctttccagagtagttcttctaataatgtaaactaatggtaaacttgttctaattgcctcccaaagcagtaggaggatgaaatggtagaagacctgtgaaagagggatctggaattttaaaaataaattcaacaccgtattaattatttgctggaaggctgcaatgtgtccaggtattagataaaaaaacggtaagcagagtctctacggaaaaaaaaaaaaaatcacaatccagcctgaaagatgagtaagagcgaggaaaaaattgaacagaactatgtagaattctataaaatttcacttatggtggagcattgtactcttagggctgcaagaaaaaaaaaatggagggcgttcttcctctctttggcttttcccaagaggcctaacgctaacaatggcaccaactactgttaataccatcaatagggaaatggtaccgcataatggatgctttgtatctctatctctcagttcagttggagctaaataaagagggcaaatgagcacccaacactgtgccaggggaaaagtgtcgcctgcaacagtgaagtcgcaggtggatgtgagatgcctgacttaggagcgcgcttaccaaggcgctaacactgctgctattatttccacccgcaccccgagcgctatgccggccgcgcctgggatgaaacacacacattgagcctacaagaccgtcctgggtctagagtgtctgtggcagccttcttttctgccccaccctgaaatcctagctatcccaggacgccctagaaggaagcccagggacggtgtggagcagcctgtactccccatctctcttccaggaggccacacccaaaacaaggccctctttgtgtctcggagaacagtggccgtatagtgctccgccggctgcccctgttaagagagagcgagcagccctcgccccggcaaccccaggcagaggcgcgtcgcggcggcggcgcaggtgggcgcaggcgcggaggtgggctctctagggccgcgcgggagccccgggtccgcacgccgcgcgcggaacacctgggggcggagccaagaccgcgtcccgcccactcccgggcgcgaagccccctccccgcgcccctcccatcgcgccgcagaggcgcgcaggtgcgtgaggccgcgcccgcccgggaccctgcagacgtgggccagccatggagcacatccgtacgcccaaggttggtgacaccagcgcgggcggaggagggacgggaggagatgggggaggaggaggagggatgctgagcgcgcgggaggccgactgctttgaggggcaccggcggagcctggaccgcgggcgagggaggagcaggcattgcctgagcatcccggggtgcctgcgagcccggtcgttctcttgctgcctcccaggcctagccttagctgctgctgggtctgacctcttggttttgggggagcgcagtggacacaagggtgaacgggagggaacctcagttgtctgctagtaactgggtgtagatcaacccttctttctcctggcacgaggctttctcttttagctgttggccgctcagagtagttgaaagggaaataagcctttcggtgacaggtgcaaggaaaacgagctaaatgcagagggactcctgcgcttggaagcttgttaaatctagggtgtcaggcccacccggctcggccttcccagtcagcatcctcatcctgagcgtagcagctgcaaggggccttacacagaacggataatcaatattcattgtaggttgaatgatggtgtgttcttgccttttccagtccgttttgttcgttagagaaaaggatgcagcttacggattcgtcacgcactgttgtgttttaacaacaccagcttttgctaattaacaaaagcaaatggtccctgatcactccagtaaattaacattggaaacgttgatcgctgtaccaaatcttcctcctcagttgtactgataatctaatttagaatgaaaatgatgatcgacgttactgcatgataaaaaccctaaacgagtgaaagaatatgcttaaaaaccctattggctgtctgttgttactaccaccacagctccttgcgtttttgcaggatgaacttccattcaaaatgtaggcccctgacaggtcaaagctaggtcagagtggccatagctcaggtggttccagggatcccacacatttaagaggggtgggggcaattgctttatggccagcaagaattgattcctaaattttggaatagttcctgagtacctttttgtaaaagcagattaaaatgatctcatgtcattggaagaagaaatcttttagtttgctggagaatgtcagttccgacagtaaatttaaattgtattgattttgcactagggaattaagttgtcgcttcacaatcatgaaattgtaaacttagaagacaatgctacaaaccacagaataggtggctcaaagctttcagagtttaagtggtactaaataatttattccagaagggtgaatttaactcatggactctgcccttgccaagggcattcttcctccttccatgatgaagggagccgtttgtaaaagtgatagctgttgtggatattgatagcaagaatgatacagtgacatggcagtggatgccactttgttagagaatatgaatttgggggagtcaaggccttttctgttctatatacaaagccacctggtacaaagtcacgtgtgaacctgagttgcaagcagtgttcttactcttaaaattggtgtttatggataccctctaagcagtgcagtacttgaagtcagaaatccttatttatctggaaatggaaacaaattgggggaaaatggaaaattgtctgaagtgttactgaattgggtgagtcattaacatttgggataaagctggtgaaaaaaataagaaattacagaggttggatggatcggattcatttattcatttattttattctacaagcatttagaacctttcatgtgccaggctctgtgttaagtgctggaagcgtccaggaactcacaatctctaaggggaggcagttgtaaatatgtcagtgtatgatagagacatgtgcaaggtgcagtgggtagagagggagactgaagagaggatcagctctgccctcaaggtcaagggaagccttcttagaagagccgtcttaacatggaaggacttaaggaggactaggagcattttcaacagtggtcatgtacttgtataaatatatattgtaataaataattacaaccctaaagaaactgaaaacaataacaatggtcaaagataaatgattccttgaggttaaataacatcctccttttgttttacatttttaagggcaaaattaattttcacagtctaaatgaaaaagagaacaacattacttacagagcttgcagagttaaatatataattgttactggtcat

SEQ ID NO: 10 - DNA, 4000 bp, Homo sapiens
agtgattggtactgctcgaaggttgccagaatgagtattgtaccgaagcccttatggttatatgactcagttataatggttcagtctctttgataccggatggctttttggaagaccatttttctgttatttaacagttgttaacaacaacaacaacaaaaagcttcctggttgtgtttgatagagtctaggggaaaaacaaagccactgttgcctcctctccatccccaaggagaatgtgggtcagggctggaggccggctctgggaatccctgagaagggagcattattaatgtcaccaccactgtgcctgctgagctgctctgtgcttcccccttgcacaagaaccaggcccagccagggaaaggaaacgcaggccattccctcagagccgaagttaagggagaaataataatacaggcacaggaggaccagcagcagccagagaggagaagtgacagggaccgaggcaaatccagtctctccccgggtttcaagaatttgagaaacacacctcttaaagatgaaatcagctgtgcgagagtgtgaggcccaggaaacctgggagtctgctgtataaatacagcaagtggctcacactcatccacccaagtgagcacttttgcaggcccagcatcttttaatggcgacaaaacaagaataaagaatgtaagtgggtgtctgaacttgaccaacattttgatgatgcgatttttccagtttcgcacactaagaggcttctgtgattttggatttgttttatatatggcagatctctagaatggtagtgttgagtctctggggttttgagcagctttgtggggggctgctgggcgggtgctgtactactgaataactatgaggttcttctaaaacatcctccgaacactctgagtttactctgaatgctaatgggattaatctgatcattttaaaggtgcatgtatgcatgctgcagggtgttcctttcccagttaattagtttgtgacccttattaagatgtctcaagtctgaggctgattaaggctgcatggtaactttgtcttttttcctaatttggaagcgcgtaaatggttaaactcctggcctgggctgggctggtgcacagcctgggcccggcgcggcgggggttaaggtgggcgcccgcgccccgcgccccgcgccctcccgccgggatgagagcgcagtccgcgccgccagcccgcccgctcgctccgaggcggcaccgggagaaagtggcggtcagggatggagctgctgccatgacaaccccggcggtcggggcccgcgcgcgtcggggctgctcccgggaggaaggcggcgcggaggccgggggcggccgctgagcttggcgtccgcgcggctccggtgcgggctgcgccgcgccttccccagcgagctaccgagcttggggccgccgcggtccgctcccgccgcccggcctctccctcctcggccaccgccgcagcccctgccccgccgagccccgccggacagcggcggccgcagcgcgcatttgggctccgaggaagttgaccgaggcggctgccgcaggatcccgggcccggatcgcacgaagcccgcgcggccgtctcctccgcgcgccacccctgcgcctcccgcgagctccacttcccatctgctattgtttccgattgttttccggtggcgagcccggctccgaaacttacaaagtgttggatgtcccccgttcgaactgagggactgcagaccgcctctgggtagctggatgaagcccaccccgtccccttctggtaccaaagtgcttactcctctccaaagtgccgtgtctgaactgccgctgggaagaagcggctcctgagacgcgcccacacctttcacctgccgcgcgcttccccctcctcggccaccttcccggcggaagcagcgaggagggagccccctttggccgtcctccgtggaaccggttttccgaggctggcaaaagccgaggctggatttgggggaggaatattagactcggaggagtctgcgcgcttttctcctccccgcgcctcccggtcgccgcgggttcaccgctcagtccccgcgctcgctccgcaccccacccacttcctgtgctcgcccggggggcgtgtgccgtgcggctgccggagttcggggaagttgtggctgtcgagaatgggggtctgtgggtacctgttcctgccctggaagtgcctcgtggtcgtgtctctcaggctgctgttccttgtacccacaggagtgcccgtgcgcagcggagatgccaccttccccaaagctatggacaacgtgacggtccggcagggggagagcgccaccctcaggtagggagctgacattgttctgcgaactgatggtttgtatggggtcggggtaaggggcaggggtgcaggtgtgtgcactgaggcgtgcctgggttggcggagaggtcgctggttccctgggctgcacaatttatggctgcgctgggggctctgcccgggaatgtggcagtcgtagggaaaggctcagaggttctggcggtgagctttttcccaaaaactggcctctgcggctcaggcacttgttaaaggtgaggggtggctggaccaggtggtcgccgagattgagggacttgtgcctggcactgtctgtgcctgagcctggtggccgtggtgacagggggcttggaggggctccccgcgagcagtcttctctgaagttaatgagccccaaaggaggggtctggcttggagtgaatgcccccactcgcccatgccatagggctttgccagccctggctcctgcactctgggagagccgctgctttgtcctgggcctgactgtgcccgggctttcctggggtgccttcatgccgtgagctggtgggcagacagagatgctttctcctgtctgaacgtggctttctgaggcccaagtcatggagtctgatttgtccgtggaaaatggcatttactgtagtgaactgtgttctgttcctgctctccaccaaaacggtacatgcaaaactcgtctactgaagagaaactaggtttcagtgttgggttgggtcctgattggcttctggggttaaggcttacaggcactgggggaggagaagaagaagaatcttggttatgctttgtgtaaggtagaatgattctatctccctgattaccttgcctgcagaaacgctaactgaatttccagtgttgataaaccacacctctcatatgcgggcaaaacacttaatgattgcgatgggaaattttattctctgggattttataagagaataagcatgaggtggacgttaagaaggttcatgggaacgatttccctgcctctccttggtttagtctgccctcctaaataaagttttccaaactaagcgacagaactaaccacaaggcaacatggcaatattcctgtcctttgcacatgaagatttctggaaagataaccctggtgctggtgtctactgttttgcccctctgatgacttcttctaggattgggttgttttggactgtatacttaaggcaatatctataggatagaaaatggtgaagaggaggcaatgtcaatacagagctgagttatcaggacattgccaaaggaagtgtgtaatttagggacccgtgcagggctacaagcatccagtgatcctttgtctaggcaaagcttaacctcatggctctggtgaactcctagttatttgttggctcacgagacccacctcttccactcttctgagcaaaaataaagcaacttccttcccccactcagaaatgattgtgtatctgctttaaaaatggatttcaggggagttacaaatatgcagtgatttcagactacttaaataaaaaaccaaaaataaatgtctagagcagtaataatcaaggaaattttcttgttcaagaaatgcttgttctctggatgccctctttgtccctagtccttggctgcaaggagggcctcccagggacagagacattctgaatggggaacattt

SEQ ID NO: 11 - DNA, 2848 bp, Homo sapiens
tttctggcattagctgcccacgtctgtggcacttcaggcccatgtaactatttccagagtgacacaagtttcttccacagttgtcaacaagtggccctcacaggttcagtgagaagaggaagagggagagagatcatcaggattaatggattacttgcatttgtgagacggtttgccaagtattgctacaaacaaggcacgggattttcttttttcttttcttttttttttgagatggagtcttgctctgtcctccaggctgtagtgcagtggagcaatcttggtttactgcattctctgcctcccaggttcaaacgattcttctgcctcagccctcccgagtagctgggattacaggcgtgtgtcacaacgccctgctaatttttgtatttttagtagagacggggttttgccatgttgcccaggctggtctggaactccctgcctcacgtgatcctcccccctcggcctcccaaagtggtgggattacaagcatgagccaccgcgcccggctaaggcatgggatgtttcgaactgctgacattagaaattcacaatccacatcattaactggatcctccatgcccactctctccctctctgcagcagcaatttcaaatctttactctccgcagttccacagaacacaagaaacaaacaaacaagcaaaaaaagtcaggcaggagcccaagtaacctctatcaaagcaaagaccagtgcctagtctaacgcttttaaggattttaaaagaggtgaaggtgtcctgcttatcctccaagcttgggtgctggggccggggcggctgagatttaccagtgaaacccaaagaaagagagggcagaaaactagagaaaagaaaccagataatgctacccaagaggacgaaataaagaagcaggaaacgaagcctgaggctaaaccctggagatgactattaggaaaacaccagaggatgccccgcccgccagcccacaatgagcagcctgtccaagtcacaaagcggggcctcgggccttgacagttcgcgatctgtaagcagaatgttccagggcctccctgtcgcctgcatccagcctgggggcaatcttcactggtgtgggaggccgaaagtggacggcgacggaggcccctctggttatctctttgccgtgccaacacagtctctgcgcccactaagatgcatgaaataaaaatttccgtgactcgccctttgcagtggagaactgaaacaggcacaccagggaattggagcggaggagggtaactcaaactcagagtgagagggtttgcagggggccgatttggggccaacaggcttcccagcaggcccccggcgcgggacagcggaaggcgaaacgctttcaagagaccccgctgccaacatccccacgccctcgcgccctcccgccgccccagaaggccaactccgcctgcctgagtcacagctggagctggggaggagccagggaaaggaggcccctgaccgtagtgcggccagcagttgcaggcagacggagcagagcggtcagggatcatgagggagagtgcgttggagcgggggcctgtgcccgaggcgccggcggggggtcccgtgcacgccgtgacggtggtgaccctgctggagaagctggcctccatgctggagactctgcgggagcggcagggaggcctggctcgaaggcagggaggcctggcagggtccgtgcgccgcatccagagcggcctgggcgctctgagtcgcagccacgacaccaccagcaacaccttggcgcagctgctggccaaggcggagcgcgtgagctcgcacgccaacgccgcccaagagcgcgcggtgcgccgcgcagcccaggtgcagcggctggaggccaaccacgggctgctggtggcgcgcgggaagctccacgttctgctcttcaaggtcagtgacctcaaacggtccccaatccgaggcctttgccggcctgtgggccaccagctgggggctccccgcttccatccacctaccacacccacattcctgacccctcccgccgtctgttgctgtggaacagactcacagagccgcacccacttcccaagacccagccccatccctccctctcacgcctgagccccgcctggccaatccaagcccgcccagctctagctcaggccacgtccgcagaatttggtctgagtcccagccaatccctaaaataacggtggttgaaagggcattccgtgactgcgggcactatcctcttctcgcccctcaccaggcctcacctactttacagcgttttgcagttcgcacgcagctttccctccccttaccttcccacgcctgcctttccccccagactctggctgcggaggtaaaaggtttcccttgtgtaattaaggagtgagtttcgggctgctgggggtaaggagctgccaggatcagtgctgtgtccgtcacatgcaggaggagggtgaagtcccagccagcgctttccagaaggcaccagagcccttgggcccggcggaccagtccgagctgggcccagagcagctggaggccgaagttggagagagctcggacgaggagccggtggagtccagggcccagcggctgcggcgcaccggattgcagaaggtacagagcctccgaagggccctttcgggccggaaaggccctgcagcgccaccgcccaccccggtcaagccgcctcgccttgggcctggccggagcgctgaagcccagccggaagcccagcctgcgctggagcccacgctggagccagagcctccgcaggacaccgaggaagatcccgggagacctggggctgccgaagaagctctgctccaaatggagagtgtagcctga

SEQ ID NO: 12 - DNA, 4000 bp, Homo sapiens
cctggcaagaatggattctctcgaaaggtttgaaaatccctattttgcttggtggcccagaccatctgtgctcaatgagctaagcaaatctggctgggctattacctgggagagtccagatttttcctctctggaggggcctgaagattatttatgggaattaattttatccccaaatctctgagaacttaaagggattgggaaggtctttctggatttccctttccctctactggagatgtagcggttcagccttcttccgatgccatgtttgtttttcgtgtcttcggcctagggtcgccttgccagcaagcctaaaggcctccaagctgacttggagggtgagggtgttttcacaaataaatacatcgcctgggcaaagggaaaatatctgtttgcaaacaaacctggaaggtggagtgagcaccatagcaaaggagggctggctttctccccggttgccccacattcagggttggagattctccactttggcattttgcagcaatggcctggcctgggattttagcagagcagtcacagagggttacacagctgctgacctcggggcatttctcctccctccatccctttctccagaccttgacttgcaggcccaagtctcttatcagaaccctagaaaaatcagtatgatgggggtacaggaggtaaggatgggaaacagaacaggactcctgacatttactccaagcaccaatattcggtgtcccaatctgggtctgctcagactgagacctactgactgtgtttgtgcttttattgacctcttcaactcaccctaaaaaaaaaaaatacatctcagagagggaaagggcaaggagaggagaccagtggagatgaaaaccctagccagtccccagtgactgtttgattattttaataaaactgggcactgccttgtgtacacctggagcaggggacgtctggtggccccactgggtggggggtgagggcccgcagcgatttcttagcatctttgatctcggcccccatcccaatgcaccttcaccctgccttcaccccagagtcgttgagagtaggggtgatgagtagggggtggaggggagatgtcaggaaggcgagcgccggccaggcggggtcaggcagctctccttctcgaggtcagcgttggagagaatgtctgcaaggctgcggaggcccgcggtgtgtttgtgtgtgtgcgtccagactcggttctctgcaccgccagcgtcactgagattacttcccgattagaagccgaccgcgtttgaaatgatttgtgcaggagtttttgcagccaccgcttgctcagagaagcagagatggatggaggttgggaaaggggtagagaggagggagttattgcaggtctgtgttgagagtcgtattgtgatttgagtgttcgggaaatctagtggaaatttggggtggggggaagggaggacgggagggtgggagggagagagaagggggagggcgacagagtgcagtgggagctagttggataggcgatttcagtactttgtgagcatcgaggcaacccaacgtcactgtgctcagctgagttggcttgtatttcagagagagagagagagggagagagagtgagagagactgactcttacctcgaatccgggaactttaatcctgaaagctgcgctcagaaaggacttcgaccattcactgggcttccaactttccctccctgggggtgtaaaggaggagcggggcactgagattatatggttgccggtgctcttggaggctattttgtgttctttggcgcttgccaactgggaagtatttagggagagcaagcgcacagcagaggaggtgtgtgttggaggtgggcagtcgccgcggaggctccagcggtaggtgcgccctagtaggcagcagtagccgctattctgggtaagcagtaaaccccgcataaaccccggagccaccatgcctgctcccccgcctcaccgccggcttccctgctaggagcagcagaggatgtggtgaatgcaccggcttcaccgaacgaggtaaccgtcccggcagatggcccgggaggctcaggagggagctcgtcggccgagtcggctggggcggcgggaatggcggattccagcccggctttgcattctgcagagcacagcttgcagagattttgcgcggctcggagctccccggcaaatggagtctgggaggccgccgcggctggcggagcggcattgaggtttgcagaagcacggcctggttctgtcaaaccgcatcttgttcgcctccgccagcccagagctccccgggaccctggcgagggcgcggggtaggattctccccgcggccggcagtgaatgggagcgcgtgtaggggcgccagccctgctttcttttgttgtgagtaggcagcggggctccagtcgccgcctccctgaagccccgagaacgaggcgaagaaagctgcttgcaagtcaggcctcagaagctgtccttctcctcggccccatttctagatctctggccacagcaggtcagggtgggatctggccgcttgcttaagcagctgctgaggttttgggggaccatcgcttgtgcccgcttcccaaagtcttcccgttctagggggaattcctacttgcgtatagaagagattggaaggagatcagagagcaggagacaggctcatcgggcttgaacagctctgcggcagttattttgtgtgttctaagctcatacgcctgcaaacccgggccgttctatgcattgcggggacccgggctgcagattcaatgtctccagcctaggacttatccgagaatgattttgtcctcgccaatcctgagcctgagcctgcagttttagcaggccaggcctggctgaagttcagagaaacccctttcggcctggtcactccacaaaatgcccgccatcccccgcccggcatcagagcgctggtggcgggcacccagtgacgagccttcctcggaacggctgcacggtgactttcttcatctagtcttctgtttggctactttttatcttttaacgaatcttacttaaggttgggataaagaaaaggatgtttaattttaaaggacttttaatgttaaggcctgtaactggtaaaaggtgtatatgaattctcttttgaacctagtctcaatctgcacaaccttccccttctgtgtttttctttttgcaagaggcgggttatttcacacatttctgcctgctgcagaaaactattcctcttgtgaggtttaataaaaagagtttcgacggcatcttgtaatttggcgaagaaagaaattctctaaaggacactgggtttttgttttgttttgtttttggttcctacccagtggcttccaaaaatacccacgccttatctttattggctcttccagaagtccagacaaatttgacgggcagcttgcttatcacggagagcctgcgcaggggagatgcgggcctcaccttctccgggtctgacgcgggtcttttgcaagaagttgtgcctgcttataaagtaatagtaatactactaggaatactagtaacagtaataattctagggccttctgcagtcaccttcggctgggaacggaggtgctggtagctggaaactgggggccaaactgctccctcctgtcactagaattgtgctctccaacctttctctcgttctctctctgtcctccccacccccatctccccctgcttcttgtcctcagagcagaaccttgcgcgggcacagggccctgggcgcaccatggccgacgcagacgagggctttggcctggcgcacacgcctctggagcctgacgcaaaagacctgccctgcgattcgaaacccgagagcgcgctcggggcccccagcaagtccccgtcgtccccgcaggccgccttcacccagcaggtaaggagacctcgcgcttcgggtccctttgcagagatcaaagtcagagtctggctttcctgctcggcttctcttgcggggacagaac

SEQ ID NO: 13 - DNA, 4000 bp, Homo sapiens
gagaaagccaaaaatttccccctaccaattacataagattccctgcttctagttagcccgcctgtagtttccccatgccagcaacttccaataagggaatacctgaagccattccttttttccactgtgaagctttccccactcttctgcctgactttcagtctgctgaatgcaagtgatgagggctgactctcttgtcatatatagcaagctctgaataatagtctttgttctcatttgaataatctttattttcacacttcttaaaaaatttaatttcctggcatgttgcataatgttaggtaagccattttctctctttgggccttactttcttcaactgaaaaactggttcaacatttattcattcttttattccgtaagccaaaaataaaattcaaagccctctgaccatatgaatggatctctcctcttggctaagggcattccaaagttaacgtgaaaaactggttcaggccataatgggaaggaggagttggacatggctcattatgctcccctaccttttgaaattcaggaccagctgaccagcattaacatcaacacagaccttaagactgatagaacagcctctttaagtctcacagactatccggtagtgtgataatgatgagaaacatttgcagtctattctctgaagcctgctacaggctccatctgcatgataaaactttggtctccacaagcccttatcttaactgagacatccctttctattgattctaagtctttatacaataacttaactctttcaaccaattgccactcagaaaatctttgaatccacctatgtcctgaaagcctcctcttccagttgtcccacctttccataccgaaccaacgtacatcttacatgtattaattgatgtcttatgtcttcctaaaatgtgtaaaaccaagttgtagcccgaccacgttgggcacatgttctcaggatctcctggggctgtggcacgggccatggtcactcatatttggctcaggataaatcccttcaaatattttacagtttgacttttcgtggacaattctacaaatattccttggcagttaaagaaataactccccaggaggtgctagacatcgggcgcatgttagaggcacaaagatgagaatgttaaaagacataaaatacaggtctgctctgggaatgcaaaaactggtaaaaggagagataaaagagcaggtgcagtctagtgaagtacccgctacctcctatcagcaaatatctgtccacctagggtgcagcgagctggagaggaaggggtggcctagagcgcaggggaaggattcctccccagccgcctgcacccctaccccggtagcggtccctgggatcgtccgtgtctccaggagaaccggaccgctctcccctccctccccgagcgagaaaggaggaccacagagatgcggcgccctccgccgtcctagagcaaccggagcggcccgagccccggcctcccggatgctggggcctggcgggtgtggagcacggggagtcgggcgtggggcgggcagggagtggagtcggggtcttactccggtggctgcagggcgcagggtagccgtgtcaggcctgcccaggtgcagagcgctcttccgcgaccccaacagcctctggtccggtctggcgcgccctcgctttcccagagggcgacctgggctatggcggccgtggcgctggcgagcgggacacgcctcggccttgtcctcgagctgctcccgggacagcccgcgctgccccgggcgcgccgggtgagtgcggggccggagcctggaagcagtcttggccctgccctgggttctaggcccggagacggggtggtgcggcggctgggaaatgggggtacaacccagagtgaggggcctcgagggacaggcagcacagcggagtcgacacccctggacctgagcctcaaggagagcagacgtgcagcggcacggggttgagccgactgctggggcagagcgcacagagtgctgtcgggggcgatgaatggccagaatttcagagctgcctttacagagctggttatgtttgagctgggtattaggttgaaaaggaatttgcaatgcaggagcaggaaggaagaactggatattcaggcaagagtagccgcaggtgcaaggacacagaacagggtgaggaaagagtttggtttcccaatgcaatggtgagaggatcggagatgagagtggtggtggctgatgatcctggccaggaaagctgggtctgtgagtagtgaatggaattgtctgtagtgcagaggaatgtggactctattaggcagacaaagttgagccagccaaagccttggagccctggagtgctggataaatagctgtggagactttctagtgcgcaaggactgaagtgcagtggaccagaatgggctcctccacagtgtggagactgagaccctgaaggaggcagtggctgagaattacgggaagtcccaacggctggaggtcagcagtatttgtttcttaagaggatgagagaaagaaggtgcaggagctgagactcctagagatatagaaaatggggacatggagattgggacgtgggtaagcaagtgaggtgggatctttgtgagagtgttgcgggtggtgggggtgcagggagtaaagtcacaacgaggatctgccctgttgagtacagtgttcagagcaacctgaatgttctgaggagccctagctgcctctgtggctggtggcagtgactggggaggacaaaggaggaagagtcctatacaggggcagcagggatggcaggaatggggacggaaggcagtgtggcataacaggcaagagccagagtcaaacaggcctgggttctgtctcagttctggaactttgggggaagttaatccctccgagtctcagtttcctcttctaaaaaacggatctgatagtaggctatgagacataacaaagaatatatgtcaagtgcttggcacaggcttaataaatgatagttgttatcaagggtgggtgacctctgaaggaggacacattgtggagagaggatgggacctagagcacagatgtggtttggggtataaggatgaaacaagaaaacttttgcagactcatgaaaaagaggagaaaatgtttgctgaaataaagatgaagagacatgagaaaattgatggctgatgccttgtctctttgtacataggaggcaaaaatcttctgctgatagagttcctgtagacattcagaatccagaatccccacaggcacccccacagtaccttttgatgccctgtctccccttcctcttggcctggtcctggggttgtcctagggcatttaaacacatgttgtttcaggagtcagtgaccttcgaggatgtggccgtctacttctctgagaacgaatggatcggcctgggccctgctcagagagccctgtacagggatgtgatgctggagaattatggggctgtggcttccctgggtaagggtctctccctttgggccctgcctccacccttgagagtttgctggctccttttttctcaaaggctcaggagttgttgataaccctcagctcaatggcagcttcaggctcttggatttttaatgacctaacctcagcagccgttggaaagtaggaagtcctggtatcagtttgggccttatacaggacttccttgctccagagtgagaggtgccaaacccctacccttgtgttgtgggtatagtgagaagagagcaaattcatggtgctccactgagccttcagttccctcccctctcggtttgcaagatccagcctaattccaagcatcctcatgaggatgtctgaacttgagagctctaagagggagaggacaggtaagaattgaggactcaattcctcaatgagtgaaatcatccatttgctgactcaaacagttactgagtcgtctgtcaacttcctgacctttgtaagtctcctggcccctctcttgtcctttcccctggaattcctt